European Patent Specification EP 4 062 951 B1, published July 23, 2025. Title: Injectable hydrogel composition having endogenous progenitor or stem cell recruitment and induction of vascular differentiation of recruited cells. Applicant: AJOU UNIVERSITY INDUSTRY-ACADEMIC COOPERATION FOUNDATION. The sequence listing filed with the application follows.

SEQUENCE LISTING (9 sequences)

SEQ ID NO: 1 - protein, 15 aa, Artificial
  vascular endothelial growth factor mimic peptide
KLTWQELYQLKYKGI

SEQ ID NO: 2 - protein, 11 aa, Artificial
  substance P
RPKPQQFFGLM

SEQ ID NO: 3 - protein, 6 aa, Artificial
  WKYMVM
WKYMVM

SEQ ID NO: 4 - DNA, 20 bp, Artificial
  vWF_Forward
cggcttgcaccattcagcta

SEQ ID NO: 5 - DNA, 25 bp, Artificial
  vWF_Reverse
tgcagaagtgagtatcacagccatc

SEQ ID NO: 6 - DNA, 24 bp, Artificial
  CD31_Forward
attgcagtggttatcatcggagtg

SEQ ID NO: 7 - DNA, 24 bp, Artificial
  CD31_Reverse
ctcgttgttggagttcagaagtgg

SEQ ID NO: 8 - DNA, 19 bp, Artificial
  GAPDH_Forward
gaaggtgaaggtcggagtc

SEQ ID NO: 9 - DNA, 20 bp, Artificial
  GAPDH_Reverse
gaagatggtgatgggatttc